European Patent Application EP 4 397 183 A2, published July 10, 2024. Title: Use of a biopolymer for reducing the formation of a biofilm. Applicant: AMSilk GmbH. Application EP. The sequence listing filed with the application follows.

SEQUENCE LISTING (8 sequences)

SEQ ID NO: 1 - protein, 24 aa, synthetic construct
  REGION 1..24: note = synthetic
  DOMAIN 1..24: note = Module A (ADF-3)
GPYGPGASAAAAAAGGYGPGSGQQ

SEQ ID NO: 2 - protein, 35 aa, synthetic construct
  REGION 1..35: note = synthetic
  DOMAIN 1..35: note = Module C (ADF-4)
GSSAAAAAAAASGPGGYGPENQGPSGPGGYGPGGP

SEQ ID NO: 3 - protein, 35 aa, synthetic construct
  REGION 1..35: note = synthetic
  DOMAIN 1..35: note = Module Cc
GSSAAAAAAAASGPGGYGPENQGPCGPGGYGPGGP

SEQ ID NO: 4 - protein, 20 aa, synthetic construct
  REGION 1..20: note = synthetic
  DOMAIN 1..20: note = Module Q (ADF-3)
GPGQQGPGQQGPGQQGPGQQ

SEQ ID NO: 5 - protein, 124 aa, synthetic construct
  REGION 1..124: note = based on ADF-3
  DOMAIN 1..124: note = NR3 (ADF-3)
GAASAAVSVGGYGPQSSSAPVASAAASRLSSPAASSRVSSAVSSLVSSGPTNQAALSNTISSVVSQVSASNPGLSGCDVLVQALLEVVSALVSILGSSSIGQINYGASAQYTQMVGQSVAQALA

SEQ ID NO: 6 - protein, 109 aa, synthetic construct
  REGION 1..109: note = based on ADF-4
  DOMAIN 1..109: note = NR4 (ADF-4)
GAYGPSPSASASVAASRLSSPAASSRVSSAVSSLVSSGPTNGAAVSGALNSLVSQISASNPGLSGCDALVQALLELVSALVAILSSASIGQVNVSSVSQSTQMISQALS

SEQ ID NO: 7 - protein, 136 aa, synthetic construct
  REGION 1..136: note = synthetic
  REGION 1..136: note = domain - derived from Latrodectus hesperus
MGQANTPWSSKANADAFINSFISAASNTGSFSQDQMEDMSLIGNTLMAAMDNMGGRITPSKLQALDMAFASSVAEIAASEGGDLGVTTNAIADALTSAFYQTTGVVNSRFISEIRSLIGMFAQASANDVYASAGSG

SEQ ID NO: 8 - protein, 137 aa, synthetic construct
  REGION 1..137: note = synthetic
  REGION 1..137: note = domain - derived from Latrodectus hesperus
MGQANTPWSSKENADAFIGAFMNAASQSGAFSSDQIDDMSVISNTLMAAMDNMGGRITQSKLQALDMAFASSVAEIAVADGQNVGAATNAISDALRSAFYQTTGVVNNQFITGISSLIGMFAQVSGNEVSYSSAGSG